European Patent Application EP 4 344 707 A1, published April 3, 2024. Title: Anti-Nectin-4 binding agent conjugates for the treatment of drug-resistant Nectin-4 associated disorders. Applicant: Emergence Therapeutics AG. Application EP. The sequence listing filed with the application follows.

SEQUENCE LISTING (112 sequences)

SEQ ID NO: 1 - protein, 8 aa, synthetic construct
  REGION 1..8: note = CDR1 VH_15A7.5 IMGT
GFTFSNYG

SEQ ID NO: 2 - protein, 8 aa, synthetic construct
  REGION 1..8: note = CDR2 VH_15A7.5 IMGT
ISNLAYGI

SEQ ID NO: 3 - protein, 12 aa, synthetic construct
  REGION 1..12: note = CDR3 VH_15A7.5 IMGT
ARGARATGWFAY

SEQ ID NO: 4 - protein, 6 aa, synthetic construct
  REGION 1..6: note = CDR1 VK_15A7.5 IMGT
QNVDTH

SEQ ID NO: 5 - skipped

SEQ ID NO: 6 - protein, 9 aa, synthetic construct
  REGION 1..9: note = CDR3 VK_15A7.5 IMGT
QQYNSYPLT

SEQ ID NO: 7 - protein, 5 aa, synthetic construct
  REGION 1..5: note = CDR1 VH_15A7.5 Kabat
NYGMA

SEQ ID NO: 8 - protein, 17 aa, synthetic construct
  REGION 1..17: note = CDR2 VH_15A7.5 Kabat
FISNLAYGINYADTVTG

SEQ ID NO: 9 - protein, 10 aa, synthetic construct
  REGION 1..10: note = CDR3 VH_15A7.5 Kabat
GARATGWFAY

SEQ ID NO: 10 - protein, 11 aa, synthetic construct
  REGION 1..11: note = CDR1 VK_15A7.5 Kabat
KASQNVDTHVA

SEQ ID NO: 11 - protein, 7 aa, synthetic construct
  REGION 1..7: note = CDR2 VK_15A7.5 Kabat
SASYRYS

SEQ ID NO: 12 - protein, 9 aa, synthetic construct
  REGION 1..9: note = CDR3 VK_15A7.5 Kabat
QQYNSYPLT

SEQ ID NO: 13 - protein, 119 aa, synthetic construct
  REGION 1..119: note = VH_15A7.5
EVKLVESGGGLVQPGGSRKLSCAASGFTFSNYGMAWVRQAPGKGPEWVAFISNLAYGINYADTVTGRFTISRENAKNTLYLEMRSLRSEDTAMYYCARGARATGWFAYWGQGTLVTVSA

SEQ ID NO: 14 - protein, 107 aa, synthetic construct
  REGION 1..107: note = VK_15A7.5
DIVMTQSQKFMSTSIGDRVSVTCKASQNVDTHVAWYQEKPGQSPKALIYSASYRYSGVPDRFTGSGSGTDFTLTISNVQSEDLADYFCQQYNSYPLTFGGGTKLEIK

SEQ ID NO: 15 - protein, 9 aa, synthetic construct
  REGION 1..9: note = CDR1 H0_15A7.5IMGT
GFTFSNYGM

SEQ ID NO: 16 - protein, 8 aa, synthetic construct
  REGION 1..8: note = CDR2 H0_15A7.5IMGT
ISNLAYGI

SEQ ID NO: 17 - protein, 12 aa, synthetic construct
  REGION 1..12: note = CDR3 H0_15A7.5IMGT
ARGARATGWFAY

SEQ ID NO: 18 - protein, 6 aa, synthetic construct
  REGION 1..6: note = CDR1 L0_15A7.5 IMGT
QNVDTH

SEQ ID NO: 19 - skipped

SEQ ID NO: 20 - protein, 9 aa, synthetic construct
  REGION 1..9: note = CDR3 L0_15A7.5 IMGT
QQYNSYPLT

SEQ ID NO: 21 - protein, 5 aa, synthetic construct
  REGION 1..5: note = CDR1 H0_15A7.5Kabat
NYGMN

SEQ ID NO: 22 - protein, 17 aa, synthetic construct
  REGION 1..17: note = CDR2 H0_15A7.5Kabat
FISNLAYGINYADSVKG

SEQ ID NO: 23 - protein, 10 aa, synthetic construct
  REGION 1..10: note = CDR3 H0_15A7.5Kabat
GARATGWFAY

SEQ ID NO: 24 - protein, 11 aa, synthetic construct
  REGION 1..11: note = CDR1 L0_15A7.5 Kabat
RASQNVDTHVA

SEQ ID NO: 25 - protein, 7 aa, synthetic construct
  REGION 1..7: note = CDR2 L0_15A7.5 Kabat
SASYLQS

SEQ ID NO: 26 - protein, 9 aa, synthetic construct
  REGION 1..9: note = CDR3 L0_15A7.5 Kabat
QQYNSYPLT

SEQ ID NO: 27 - protein, 119 aa, synthetic construct
  REGION 1..119: note = H0_15A7.5
EVQLVESGGGLVQPGGSLRLSCAASGFTFSNYGMNWVRQAPGKGLEWVSFISNLAYGINYADSVKGRFTISRDNAKNSLYLQMNSLRAEDTAVYYCARGARATGWFAYWGQGTLVTVSS

SEQ ID NO: 28 - protein, 107 aa, synthetic construct
  REGION 1..107: note = L0_15A7.5
DIQMTQSPSSLSASVGDRVTITCRASQNVDTHVAWFQQKPGKAPKSLIYSASYLQSGVPSRFSGSGSGTDFTLTISSLQPEDFATYYCQQYNSYPLTFGGGTKVEIK

SEQ ID NO: 29 - protein, 8 aa, synthetic construct
  REGION 1..8: note = CDR1 H1_15A7.5 IMGT
GFTFSNYG

SEQ ID NO: 30 - protein, 8 aa, synthetic construct
  REGION 1..8: note = CDR2 H1_15A7.5 IMGT
ISNLAYGI

SEQ ID NO: 31 - protein, 12 aa, synthetic construct
  REGION 1..12: note = CDR3 H1_15A7.5 IMGT
ARGARATGWFAY

SEQ ID NO: 32 - protein, 6 aa, synthetic construct
  REGION 1..6: note = CDR1 L1_15A7.5 IMGT
QNVDTH

SEQ ID NO: 33 - skipped

SEQ ID NO: 34 - protein, 9 aa, synthetic construct
  REGION 1..9: note = CDR3 L1_15A7.5 IMGT
QQYNSYPLT

SEQ ID NO: 35 - protein, 5 aa, synthetic construct
  REGION 1..5: note = CDR1 H1_15A7.5 Kabat
NYGMA

SEQ ID NO: 36 - protein, 17 aa, synthetic construct
  REGION 1..17: note = CDR2 H1_15A7.5 Kabat
FISNLAYGINYADTVTG

SEQ ID NO: 37 - protein, 10 aa, synthetic construct
  REGION 1..10: note = CDR3 H1_15A7.5 Kabat
GARATGWFAY

SEQ ID NO: 38 - protein, 11 aa, synthetic construct
  REGION 1..11: note = CDR1 L1_15A7.5 Kabat
KASQNVDTHVA

SEQ ID NO: 39 - protein, 7 aa, synthetic construct
  REGION 1..7: note = CDR2 L1_15A7.5 Kabat
SASYRYS

SEQ ID NO: 40 - protein, 9 aa, synthetic construct
  REGION 1..9: note = CDR3 L1_15A7.5 Kabat
QQYNSYPLT

SEQ ID NO: 41 - protein, 119 aa, synthetic construct
  REGION 1..119: note = H1_15A7.5
EVQLVESGGGLVQPGGSLRLSCAASGFTFSNYGMAWVRQAPGKGLEWVSFISNLAYGINYADTVTGRFTISRDNAKNSLYLQMNSLRAEDTAVYYCARGARATGWFAYWGQGTLVTVSS

SEQ ID NO: 42 - protein, 108 aa, synthetic construct
  REGION 1..108: note = L1_15A7.5
DIQMTQSPSSLSASVGDRVTITCCKASQNVDTHVAWFQQKPGKAPKSLIYSASYRYSGVPSRFSGSGSGTDFTLTISSLQPEDFATYYCQQYNSYPLTFGGGTKVEIK

SEQ ID NO: 43 - protein, 8 aa, synthetic construct
  REGION 1..8: note = CDR1 H2_15A7.5 IMGT
GFTFSNYG

SEQ ID NO: 44 - protein, 8 aa, synthetic construct
  REGION 1..8: note = CDR2 H2_15A7.5 IMGT
ISNLAYGI

SEQ ID NO: 45 - protein, 12 aa, synthetic construct
  REGION 1..12: note = CDR3 H2_15A7.5 IMGT
ARGARATGWFAY

SEQ ID NO: 46 - protein, 6 aa, synthetic construct
  REGION 1..6: note = CDR1 L2_15A7.5 IMGT
QNVDTH

SEQ ID NO: 47 - skipped

SEQ ID NO: 48 - protein, 9 aa, synthetic construct
  REGION 1..9: note = CDR3 L2_15A7.5 IMGT
QQYNSYPLT

SEQ ID NO: 49 - protein, 5 aa, synthetic construct
  REGION 1..5: note = CDR1 H2_15A7.5 Kabat
NYGMA

SEQ ID NO: 50 - protein, 17 aa, synthetic construct
  REGION 1..17: note = CDR2 H2_15A7.5 Kabat
FISNLAYGINYADTVTG

SEQ ID NO: 51 - protein, 10 aa, synthetic construct
  REGION 1..10: note = CDR3 H2_15A7.5 Kabat
GARATGWFAY

SEQ ID NO: 52 - protein, 11 aa, synthetic construct
  REGION 1..11: note = CDR1 L2_15A7.5 Kabat
KASQNVDTHVA

SEQ ID NO: 53 - protein, 7 aa, synthetic construct
  REGION 1..7: note = CDR2 L2_15A7.5 Kabat
SASYRYS

SEQ ID NO: 54 - protein, 9 aa, synthetic construct
  REGION 1..9: note = CDR3 L2_15A7.5 Kabat
QQYNSYPLT

SEQ ID NO: 55 - protein, 119 aa, synthetic construct
  REGION 1..119: note = H2_15A7.5
EVQLVESGGGLVQPGGSLRLSCAASGFTFSNYGMAWVRQAPGKGLEWVAFISNLAYGINYADTVTGRFTISRDNAKNSLYLQMNSLRAEDTAVYYCARGARATGWFAYWGQGTLVTVSS

SEQ ID NO: 56 - protein, 107 aa, synthetic construct
  REGION 1..107: note = L2_15A7.5
DIQMTQSPSSLSASVGDRVTITCKASQNVDTHVAWYQQKPGKAPKALIYSASYRYSGVPSRFSGSGSGTDFTLTISSLQPEDFATYYCQQYNSYPLTFGGGTKVEIK

SEQ ID NO: 57 - protein, 8 aa, synthetic construct
  REGION 1..8: note = CDR1 H3_15A7.5 IMGT
GFTFSNYG

SEQ ID NO: 58 - protein, 8 aa, synthetic construct
  REGION 1..8: note = CDR2 H3_15A7.5 IMGT
ISNLAYGI

SEQ ID NO: 59 - protein, 12 aa, synthetic construct
  REGION 1..12: note = CDR3 H3_15A7.5 IMGT
ARGARATGWFAY

SEQ ID NO: 60 - protein, 6 aa, synthetic construct
  REGION 1..6: note = CDR1 L3_15A7.5 IMGT
QNVDTH

SEQ ID NO: 61 - skipped

SEQ ID NO: 62 - protein, 9 aa, synthetic construct
  REGION 1..9: note = CDR3 L3_15A7.5 IMGT
QQYNSYPLT

SEQ ID NO: 63 - protein, 5 aa, synthetic construct
  REGION 1..5: note = CDR1 H3_15A7.5 Kabat
NYGMA

SEQ ID NO: 64 - protein, 17 aa, synthetic construct
  REGION 1..17: note = CDR2 H3_15A7.5 Kabat
FISNLAYGINYADTVTG

SEQ ID NO: 65 - protein, 10 aa, synthetic construct
  REGION 1..10: note = CDR3 H3_15A7.5 Kabat
GARATGWFAY

SEQ ID NO: 66 - protein, 11 aa, synthetic construct
  REGION 1..11: note = CDR1 L3_15A7.5 Kabat
KASQNVDTHVA

SEQ ID NO: 67 - protein, 7 aa, synthetic construct
  REGION 1..7: note = CDR2 L3_15A7.5 Kabat
SASYRYS

SEQ ID NO: 68 - protein, 9 aa, synthetic construct
  REGION 1..9: note = CDR3 L3_15A7.5 Kabat
QQYNSYPLT

SEQ ID NO: 69 - protein, 119 aa, synthetic construct
  REGION 1..119: note = H3_15A7.5
EVQLVESGGGLVQPGGSLRLSCAASGFTFSNYGMAWVRQAPGKGPEWVAFISNLAYGINYADTVTGRFTISRDNAKNSLYLQMNSLRAEDTAVYYCARGARATGWFAYWGQGTLVTVSS

SEQ ID NO: 70 - protein, 108 aa, synthetic construct
  REGION 1..108: note = L3_15A7.5
DIQMTQSPSSLSASVGDRVTITCKASQNVDTHVAWYYQQKPGKSPKALIYSASYRYSGVPSRFSGSGSGTDFTLTISSLQPEDFATYYCQQYNSYPLTFGGGTKVEIK

SEQ ID NO: 71 - protein, 107 aa, synthetic construct
  REGION 1..107: note = L3_15A7.5_mod
DIQMTQSPSSLSASVGDRVTITCKASQNVDTHVAWYYQQKPGKSPKALIYSASYRYSGVPSRFSGSGSGTDFTLTISSLQPEDFATYCQQYNSYPLTFGGGTKVEIK

SEQ ID NO: 72 - protein, 8 aa, synthetic construct
  REGION 1..8: note = CDR1 VH_HA22
GFTFSSYN

SEQ ID NO: 73 - protein, 8 aa, synthetic construct
  REGION 1..8: note = CDR2 VH_HA22
ISSSSSTI

SEQ ID NO: 74 - protein, 10 aa, synthetic construct
  REGION 1..10: note = CDR3 VH_HA22
ARAYYYGMDV

SEQ ID NO: 75 - protein, 6 aa, synthetic construct
  REGION 1..6: note = CDR1 VK_HA22
QGISGW

SEQ ID NO: 76 - skipped

SEQ ID NO: 77 - protein, 9 aa, synthetic construct
  REGION 1..9: note = CDR3 VK_HA22
QQANSFPPT

SEQ ID NO: 78 - protein, 117 aa, synthetic construct
  REGION 1..117: note = VH_HA22
EVQLVESGGGLVQPGGSLRLSCAASGFTFSSYNMNWVRQAPGKGLEWVSYISSSSSTIYYADSVKGRFTISRDNAKNSLSLQMNSLRDEDTAVYYCARAYYYGMDVWGQGTTVTVSS

SEQ ID NO: 79 - protein, 107 aa, synthetic construct
  REGION 1..107: note = VK_HA22
DIQMTQSPSSVSASVGDRVTITCRASQGISGWLAWYQQKPGKAPKFLIYAASTLQSGVPSRFSGSGSGTDFTLTISSLQPEDFATYYCQQANSFPPTFGGGTKVEIK

SEQ ID NO: 80 - protein, 8 aa, synthetic construct
  REGION 1..8: note = CDR1 VH_5A12.2
GFTFNSMY

SEQ ID NO: 81 - protein, 8 aa, synthetic construct
  REGION 1..8: note = CDR2 VH_5A12.2
IYAGTGGT

SEQ ID NO: 82 - protein, 13 aa, synthetic construct
  REGION 1..13: note = CDR3 VH_5A12.2
AIRSGFVPMDYWG

SEQ ID NO: 83 - protein, 118 aa, synthetic construct
  REGION 1..118: note = VH_5A12.2
QIQLQQSGAELVKPGASVTLSCKTSGFTFNSMYISWLKQKPGQSLEWIAWIYAGTGGTRFNQKFTGKVQLTVDTSSSTAYMQFSSLTTDDSAIYYCAIRSGFVPMDYWGQGTSVTVSS

SEQ ID NO: 84 - protein, 6 aa, synthetic construct
  REGION 1..6: note = CDR1 VK_5A12.2
QSVSND

SEQ ID NO: 85 - skipped

SEQ ID NO: 86 - protein, 6 aa, synthetic construct
  REGION 1..6: note = CDR3 VK_5A12.2
QQDYSS

SEQ ID NO: 87 - protein, 107 aa, synthetic construct
  REGION 1..107: note = VK_5A12.2
SIVMTQTPKFLLVSAGDRVTITCKASQSVSNDVAWYQQKPGQSPKLLIYYASNRYTGVPDRFTGSGYGTDFTFTISTVQAEDLAVYFCQQDYSSPWTFGGGTKLEIK

SEQ ID NO: 88 - protein, 8 aa, synthetic construct
  REGION 1..8: note = CDR1 VH_9A2.7
GYNFTTFW

SEQ ID NO: 89 - protein, 8 aa, synthetic construct
  REGION 1..8: note = CDR2 VH_9A2.7
IYPSDSYA

SEQ ID NO: 90 - protein, 13 aa, synthetic construct
  REGION 1..13: note = CDR3 VH_9A2.7
TRPSYFGRNSFAY

SEQ ID NO: 91 - protein, 120 aa, synthetic construct
  REGION 1..120: note = VH_9A2.7
QVQLQQPGAELVRPGASVKLSCKASGYNFTTFWINWVKQRPGQGLEWIGNIYPSDSYANYNQKFKDKATLTVDKSSTTAYMQLSSPTSEDSAVYYCTRPSYFGRNSFAYWGQGTLVTVSA

SEQ ID NO: 92 - protein, 12 aa, synthetic construct
  REGION 1..12: note = CDR1 VK_9A2.7
QSLLYSVNHKNY

SEQ ID NO: 93 - skipped

SEQ ID NO: 94 - protein, 9 aa, synthetic construct
  REGION 1..9: note = CDR3 VK_9A2.7
HQYYTYPLT

SEQ ID NO: 95 - protein, 113 aa, synthetic construct
  REGION 1..113: note = VK_9A2.7
DIVMTQSPSSLVVSVGEKVTMSCKSSQSLLYSVNHKNYLAWYQQKPGQSPKLLIYWASTRESGVPDRFTGSGSGTDFSLTISSVKAEDLAVYYCHQYYTYPLTFGAGTKLELK

SEQ ID NO: 96 - protein, 8 aa, synthetic construct
  REGION 1..8: note = CDR1 VH_3A1.4
GDSITSGY

SEQ ID NO: 97 - protein, 7 aa, synthetic construct
  REGION 1..7: note = CDR2 VH_3A1.4
ISNSGIT

SEQ ID NO: 98 - protein, 15 aa, synthetic construct
  REGION 1..15: note = CDR3 VH_3A1.4
TRFGSTMILYYTMDY

SEQ ID NO: 99 - protein, 121 aa, synthetic construct
  REGION 1..121: note = VH_3A1.4
DVQLQESGPSLVKPSQTLSLTCSVTGDSITSGYWNWIRKFPGNKLEYMGYISNSGITYYNPSLKSRISITRDTSKNQYFLQLNSVTAEDTATYYCTRFGSTMILYYTMDYWGQGTSVTVSS

SEQ ID NO: 100 - protein, 6 aa, synthetic construct
  REGION 1..6: note = CDR1 VK_3A1.4
QSISDY

SEQ ID NO: 101 - skipped

SEQ ID NO: 102 - protein, 9 aa, synthetic construct
  REGION 1..9: note = CDR3 VK_3A1.4
QNGHSFPLT

SEQ ID NO: 103 - protein, 107 aa, synthetic construct
  REGION 1..107: note = VK_3A1.4
DIVMTQSPVTLSVTPGDRVSLSCRASQSISDYLHWYQQKSQESPRLLIKYASKSISGIPSRFSGSGSGSNFTLSINSVEPEDVGVYYCQNGHSFPLTFGAGTKLELK

SEQ ID NO: 104 - protein, 8 aa, synthetic construct
  REGION 1..8: note = CDR1 VH_8F06
GYTFTSYV

SEQ ID NO: 105 - protein, 8 aa, synthetic construct
  REGION 1..8: note = CDR2 VH_8F06
INPYNDGT

SEQ ID NO: 106 - protein, 6 aa, synthetic construct
  REGION 1..6: note = CDR3 VH_8F06
VTLFAY

SEQ ID NO: 107 - protein, 113 aa, synthetic construct
  REGION 1..113: note = VH_8F06
EVQLQQSGPELVKPGASVKMSCKASGYTFTSYVMHWVKQKPGQGLEWIGYINPYNDGTKYNEKFKGKATLTSDKSSSTAYMELSSLTSEDSAVYYCVTLFAYWGQGTLVTVSA

SEQ ID NO: 108 - protein, 5 aa, synthetic construct
  REGION 1..5: note = CDR1 VK_8F06
SSISY

SEQ ID NO: 109 - skipped

SEQ ID NO: 110 - protein, 9 aa, synthetic construct
  REGION 1..9: note = CDR3 VK_8F06
HQRSSYPFT

SEQ ID NO: 111 - protein, 106 aa, synthetic construct
  REGION 1..106: note = VK_8F06
QIVLTQSPAIMSASPGEKVTMTCSASSSISYMHWYQQKPGTSPKRWIYDTSKLASGVPARFSGSGSGTSYSLTISSMEAEDAATYYCHQRSSYPFTFGSGTKLEIK

SEQ ID NO: 112 - protein, 510 aa, Human
MPLSLGAEMWGPEAWLLLLLLLASFTGRCPAGELETSDVVTVVLGQDAKLPCFYRGDSGEQVGQVAWARVDAGEGAQELALLHSKYGLHVSPAYEGRVEQPPPPRNPLDGSVLLRNAVQADEGEYECRVSTFPAGSFQARLRLRVLVPPLPSLNPGPALEEGQGLTLAASCTAEGSPAPSVTWDTEVKGTTSSRSFKHSRSAAVTSEFHLVPSRSMNGQPLTCVVSHPGLLQDQRITHILHVSFLAEASVRGLEDQNLWHIGREGAMLKCLSEGQPPPSYNWTRLDGPLPSGVRVDGDTLGFPPLTTEHSGIYVCHVSNEFSSRDSQVTVDVLDPQEDSGKQVDLVSASVVVVGVIAALLFCLLVVVVVLMSRYHRRKAQQMTQKYEEELTLTRENSIRRLHSHHTDPRSQPEESVGLRAEGHPDSLKDNSSCSVMSEEPEGRSYSTLTTVREIETQTELLSPGSGRAEEEEDQDEGIKQAMNHFVQENGTLRAKPTGNGIYINGRGHLV